European Patent Application EP 4 553 166 A1, published May 14, 2025. Title: METHOD FOR PREPARING A SAMPLE FOR ANALYSIS. Applicant: MinervaX ApS. The sequence listing filed with the application follows.

SEQUENCE LISTING (6 sequences)

SEQ ID NO: 1 - protein, 235 aa, synthetic construct
GQQMETGDQRFGDLVFRQLAPNVWQHTSYLDMPGFGAVASNGLIVRDGGRVLVVDTAWTDDQTAQILNWIKQEINLPVALAVVTHAHQDKMGGMDALHAAGIATYANALSNQLAPQEGMVAAQHSLTFAANGWVEPATAPNFGPLKVFYPGPGHTSDNITVGIDGTDIAFGGCLIKDSKAKSLGNLGDADTEHYAASARAFGAAFPKASMIVMSHSAPDSRAAITHTARMADKLR

SEQ ID NO: 2 - protein, 280 aa, synthetic construct
MKYLLPTAAAGLLLLAAQPAMAMAAHHHHHHSSGVDLGTENLYFQGQQMETGDQRFGDLVFRQLAPNVWQHTSYLDMPGFGAVASNGLIVRDGGRVLVVDTAWTDDQTAQILNWIKQEINLPVALAVVTHAHQDKMGGMDALHAAGIATYANALSNQLAPQEGMVAAQHSLTFAANGWVEPATAPNFGPLKVFYPGPGHTSDNITVGIDGTDIAFGGCLIKDSKAKSLGNLGDADTEHYAASARAFGAAFPKASMIVMSHSAPDSRAAITHTARMADKLR

SEQ ID NO: 3 - protein, 255 aa, synthetic construct
HHHHHHSSGVDLGTENLYFQGQQMETGDQRFGDLVFRQLAPNVWQHTSYLDMPGFGAVASNGLIVRDGGRVLVVDTAWTDDQTAQILNWIKQEINLPVALAVVTHAHQDKMGGMDALHAAGIATYANALSNQLAPQEGMVAAQHSLTFAANGWVEPATAPNFGPLKVFYPGPGHTSDNITVGIDGTDIAFGGCLIKDSKAKSLGNLGDADTEHYAASARAFGAAFPKASMIVMSHSAPDSRAAITHTARMADKLR

SEQ ID NO: 4 - protein, 270 aa, Klebsiella sp.
MELPNIMHPVAKLSTALAAALMLSGCMPGEIRPTIGQQMETGDQRFGDLVFRQLAPNVWQHTSYLDMPGFGAVASNGLIVRDGGRVLVVDTAWTDDQTAQILNWIKQEINLPVALAVVTHAHQDKMGGMDALHAAGIATYANALSNQLAPQEGMVAAQHSLTFAANGWVEPATAPNFGPLKVFYPGPGHTSDNITVGIDGTDIAFGGCLIKDSKAKSLGNLGDADTEHYAASARAFGAAFPKASMIVMSHSAPDSRAAITHTARMADKLR

SEQ ID NO: 5 - protein, 347 aa, synthetic construct
MAEVISGSAVTLNTNMTKNVQNGRAYIDLYDVKNGKIDPLQLITLNSPDLKAQYVIRQGGNYFTQPSELTTVGAASINYTVLKTDGSPHTKPDGQVDIINVSLTIYNSSALRDKIDEVKKKAEDPKWDEGSRDKVLISLDDIKTDIDNNPKTQSDIANKITEVTNLEKILVPRIPEFSTIPGSAATLNTSITKNIQNGNAYIDLYDVKLGKIDPLQLIVLEQGFTAKYVFRQGTKYYGDVSQLQSTGRASLTYNIFGEDGLPHVKTDGQIDIVSVALTIYDSTTLRDKIEEVRTNANDPKWTEESRTEVLTGLDTIKTDIDNNPKTQTDIDSKIVEVNELEKLLVLS

SEQ ID NO: 6 - protein, 347 aa, synthetic construct
MAEVISGSAATLNSALVKNVSGGKAYIDIYDVKNGKIDPLNLIVLTPSNYSANYYIKQGGRIFTSVNQLQTPGTATITYNILDENGNPYTKSDGQIDIVSLVTTVYDTTELRNNINKVIENANDPKWSDDSRKDVLSKIEVIKNDIDNNPKTQSDIDNKIVEVNELEKLLVLPEFSTIPGSAATLNTSITKNIQNGNAYIDLYDVKNGLIDPQNLIVLNPSSYSANYYIKQGAKYYSNPSEITTTGSATITFNILDETGNPHKKADGQIDIVSVNLTIYDSTALRNRIDEVINNANDPKWSDGSRDEVLTGLEKIKKDIDNNPKTQIDIDNKINEVNEIEKLLVVSL